European Patent Specification EP 4 029 938 B1, published January 28, 2026. Title: Nucleic Acids detection method using real-time PCR. Applicant: SEKISUI MEDICAL CO., LTD. The sequence listing filed with the application follows.

SEQUENCE LISTING (12 sequences)

SEQ ID NO: 1 - DNA, 20 bp, Artificial Sequence
  primer
ccctttcaaccatgctgaca

SEQ ID NO: 2 - DNA, 20 bp, Artificial Sequence
  primer
gtgccagctgcagggtttag

SEQ ID NO: 3 - DNA, 19 bp, Artificial Sequence
  primer
cagctcagcgcccattacg

SEQ ID NO: 4 - DNA, 18 bp, Artificial Sequence
  primer
tgggactccaggagccag

SEQ ID NO: 5 - DNA, 18 bp, Artificial Sequence
  primer
gcggagggaagctcatca

SEQ ID NO: 6 - DNA, 17 bp, Artificial Sequence
  primer
gtctgacctcgcgcgga

SEQ ID NO: 7 - DNA, 27 bp, Artificial Sequence
  probe
cctctggtttttgtaaaggtgcccact

SEQ ID NO: 8 - DNA, 21 bp, Artificial Sequence
  probe
tctgcacgggcagcaggttgg

SEQ ID NO: 9 - DNA, 21 bp, Artificial Sequence
  probe
ccacgagctgagtgcgtcctg

SEQ ID NO: 10 - DNA, 503 bp, Homo sapiens
gactgaattcggctctgtctagtgtgataacattttgttatcttattcattgtcttcatccctgaaatacactctgctctctcctatctctgctctgaaaggcagaaagagggcagccctctccaaggcaaaatggggctcctgtggggaacagaggggtgcctctgtcaacaaaggtgatgccacatccctttcaaccatgctgacacctctggtttttgtaaaggtgcccactcctgtgcacggtgatgcataggcacctgcaccccgtgcctaaaccctgcagctggcacgggccctgtctgctcttcattcaccgttctcacgagttgcaataagttcagccctccatgtcacactgtgttttccatcctggggagtgtttcacagctatcccaagccccacgctgacgaatcacggccgaaaacacactctgatgccagcacagaccacggagcaaatgtcagacaagatcagcctcggaaaagtgaggaattcagtc

SEQ ID NO: 11 - DNA, 421 bp, Homo sapiens
gctttaaattatttacaatcccctaatggaaattttcactaatgagatatcataatgaatgtgaattttatttctgaaatctctaataaatcagtcttctccctggttttcccagctcagcgcccattacgtttctgttctctttcccttagtggcattatttgtatcactgtgcatcagcacagtgtgcgctgccaacctgctgcccgtgcagaaactctagggtaagagctggctcctggagtcccacccaggctgcgtgtccctcacagtctgctctgtgtctatgtgtgtgtgttggggggatattattggacaattcaagggaggctcagtgaggaggaaggaaaatttcatgtaattctttctggtttgtctttctcaaccccctcctcctgcctactccttaactgagagagtg

SEQ ID NO: 12 - DNA, 341 bp, Homo sapiens
atagggcggagggaagctcatcagtggggccacgagctgagtgcgtcctgtcactccactcccatgtcccttgggaaggtctgagactagggccagaggcggccctaacagggctctccctgagcttcggggaggtgagttcccagagaacggggctccgcgcgaggtcagactgggcaggagatgccgtggaccccgcccttcggggaggggcccggcggatgcctcctttgccggagcttggaacagactcacggccagcgaagtgagttcaatggctgaggtgaggtaccccgcaggggacctcataacccaattcagactactctcctccgcccatt